European Patent Specification EP 3 741 376 B1, published September 24, 2025. Title: PROBIOTICS FOR INHIBITING OR PREVENTING PROGRESSION OF KIDNEY DISEASE AND COMPOSITION FOR INHIBITING OR PREVENTING PROGRESSION OF KIDNEY DISEASE COMPRISING THE SAME. Applicant: GREEN CROSS WellBeing Corporation. The sequence listing filed with the application follows.

SEQUENCE LISTING (2 sequences)

SEQ ID NO: 1 - RNA, 1442 nt, Artificial Sequence
  16S rRNA of bacterial strain, L. acidophilus BP105
ctcaggacgaacgctggcggcgtgcctaatacatgcaagtcgagcgagctgaaccaacagattcacttcggtgatgacgttgggaacgcgagcggcggatgggtgagtaacacgtggggaacctgccccatagtctgggataccacttggaaacaggtgctaataccggataagaaagcagatcgcatgatcagcttataaaaggcggcgtaagctgtcgctatgggatggccccgcggtgcattagctagttggtagggtaacggcctaccaaggcaatgatgcatagccgagttgagagactgatcggccacattgggactgagacacggcccaaactcctacgggaggcagcagtagggaatcttccacaatggacgaaagtctgatggagcaacgccgcgtgagtgaagaaggttttcggatcgtaaagctctgttgttggtgaagaaggatagaggtagtaactggcctttatttgacggtaatcaaccagaaagtcacggctaactacgtgccagcagccgcggtaatacgtaggtggcaagcgttgtccggatttattgggcgtaaagcgagcgcaggcggaagaataagtctgatgtgaaagccctcggcttaaccgaggaactgcatcggaaactgtttttcttgagtgcagaagaggagagtggaactccatgtgtagcggtggaatgcgtagatatatggaagaacaccagtggcgaaggcggctctctggtctgcaactgacgctgaggctcgaaagcatgggtagcgaacaggattagataccctggtagtccatgccgtaaacgatgagtgctaagtgttgggaggtttccgcctctcagtgctgcagctaacgcattaagcactccgcctggggagtacgaccgcaaggttgaaactcaaaggaattgacgggggcccgcacaagcggtggagcatgtggtttaattcgaagcaacgcgaagaaccttaccaggtcttgacatctagtgcaatccgtagagatacggagttcccttcggggacactaagacaggtggtgcatggctgtcgtcagctcgtgtcgtgagatgttgggttaagtcccgcaacgagcgcaacccttgtcattagttgccagcattaagttgggcactctaatgagactgccggtgacaaaccggaggaaggtggggatgacgtcaagtcatcatgccccttatgacctgggctacacacgtgctacaatggacagtacaacgaggagcaagcctgcgaaggcaagcgaatctcttaaagctgttctcagttcggactgcagtctgcaactcgactgcacgaagctggaatcgctagtaatcgcggatcagcacgccgcggtgaatacgttcccgggccttgtacacaccggcccgtcacaccatgggaagtctgcaatgccccaaacccgg

SEQ ID NO: 2 - RNA, 1401 nt, Artificial Sequence
  16S rRNA of bacterial strain, L.salivarius BP121
cctagatatagtttttttaatgctcaggacgaacgctggcggcgtgcctaatacatgcaagtcgaacgaaactttcttacaccgaatgcttgcattcatcgtaagaagttgagtggcggacgggtgagtaacacgtgggtaacctgcctaaaagaaggggataacacttggaaacaggtgctaataccgtatatctctaaggatcgcatgatccttagatgaaagatggttctgctatcgcttttagatggacccgcggcgtattaactagttggtggggtaacggcctaccaaggtgatgatacgtagccgaactgagaggttgatcggccacattgggactgagacacggcccaaactcctacgggaggcagcagtagggaatcttccacaatggacgcaagtctgatggagcaacgccgcgtgagtgaagaaggtcttcggatcgtaaaactctgttgttagagaagaacacgagtgagagtaactgttcattcgatgacggtatctaaccagcaagtcacggctaactacgtgccagcagccgcggtaatacgtaggtggcaagcgttgtccggatttattgggcgtaaagggaacgcaggcggtcttttaagtctgatgtgaaagccttcggcttaaccggagtagtgcattggaaactggaagacttgagtgcagaagaggagagtggaactccatgtgtagcggtgaaatgcgtagatatatggaagaacaccagtggcgaaagcggctctctggtctgtaactgacgctgaggttcgaaagcgtgggtagcaaacaggattagataccctggtagtccacgccgtaaacgatgaatgctaggtgttggagggtttccgcccttcagtgccgcagctaacgcaataagcattccgcctggggagtacgaccgcaaggttgaaactcaaaggaattgacgggggcccgcacaagcggtggagcatgtggtttaattcgaagcaacgcgaagaaccttaccaggtcttgacatcctttgaccacctaagagattaggctttcccttcggggacaaagtgacaggtggtgcatggctgtcgtcagctcgtgtcgtgagatgttgggttaagtcccgcaacgagcgcaacccttgttgtcagttgccagcattaagttgggcactctggcgagactgccggtgacaaaccggaggaaggtggggacgacgtcaagtcatcatgccccttatgacctgggctacacacgtgctacaatggacggtacaacgagtcgcgagaccgcgaggtttagctaatctcttaaagccgttctcagttcggattgtaggctgcaactcgcctacatgaagtcggaatcgctagtaatcgcgaatcagcatgtcgcggtgaatacgtt